European Patent Application EP 4 190 903 A1, published June 7, 2023. Title: Enzymatic agent for catalyzing epimerization of sugars. Applicant: Nihon Shokuhin Kako Co., Ltd. The sequence listing filed with the application follows.

SEQUENCE LISTING (12 sequences)

SEQ ID NO: 1 - protein, 452 aa, Lunatimonas lonarensis
MNKPIIIVLFSCLCGLAALVSCRNSESESVRLRYADTLEAVVLDNILTKWYPAAYDYQDGGYISSFEFDFSPSERQNKMIVSQARHLWTTSKAALDYPEVDHYREGAELGFRFLRDRFWDKEHGGFHTLLSKEGEVITSGPDAKTAYGNAFAIYGLAAYYAMSNNEEVLSLAQKAFMWLEKNSYDPEFGGYFQNLGVDGTPLRRTDETPSTSTIGYKDQNSSIHLLEAFTELYHVWKDPLLKTRLEELLEIIRDKIVQPEGYLQLFLYPDFTPVSFRDSSAAVIEKHHAIDHVSYGHDVETAYLMMEASEALGRPHDEKTWAVGKKMVDHALKFGWDNEKGGFYDGGYYFKGEEIPRVVKDTKNWWAQAEGLNTLLIMADLYPDDDWGYFSKFELQWDYIDKYLIDHEHGEWYAGGIDMQPHFKTSQKGHIWKTAYHNYRSLANCIKRLREN

SEQ ID NO: 2 - DNA, 1359 bp, Lunatimonas lonarensis
atgaacaaaccgatcatcatcgttctgtttagctgcctgtgtggacttgcagcgttagtgtcttgcagaaattcagaaagcgaatctgtcagacttcgctatgcagatacattagaagcggttgtgctggataacatccttacaaaatggtatccggctgcctatgattatcaagatggcggatacatttcaagctttgaatttgatttttcaccgagcgaaagacaaaacaaaatgatcgtttctcaggcacgccatctttggacaacatcaaaagcagcgttagattatccggaagtggatcattatagagaaggcgcggaattaggatttcgctttctgagagatcgcttttgggataaagaacatggcggatttcatacactgctttcaaaagaaggcgaagtgatcacaagcggaccggatgctaaaacagcctatggcaatgcttttgccatttatggattagctgcctattatgctatgagcaataacgaagaagtgctttctttagcacaaaaagcgtttatgtggctggagaaaaatagctatgatccggaatttggcggatattttcagaacctgggcgtcgatggaacaccgcttagacgcacagatgaaacaccgtctacatcaacaatcggatacaaagatcagaactcttcaatccatttactggaagcgtttacagaactgtatcatgtctggaaagatccgcttttaaaaacaagacttgaagaactgcttgaaatcattcgcgataaaattgttcaaccggaaggatatctgcagctgtttctgtatccggattttacaccggtctcttttagagatagctctgcagcggttatcgaaaaacatcatgctatcgatcatgtttcatatggccatgatgtggaaacagcctatctgatgatggaagctagcgaagcccttggcagaccgcatgatgaaaaaacatgggcagtgggcaagaaaatggtcgatcatgcgcttaaatttggctgggataatgaaaaaggcggattttacgatggcggatactactttaaaggcgaagaaattccgagagtcgttaaagatacaaaaaattggtgggcacaagcggaaggattaaacacattactgatcatggctgatctgtatccggatgatgattggggctattttagcaaatttgaacttcagtgggattacatcgataaatacctgatcgatcatgaacatggagaatggtatgccggcggaatcgatatgcaaccgcattttaaaacatctcagaaaggccatatctggaaaacagcttaccataactaccgctcactggccaactgtattaaaagactgcgcgaaaattaa

SEQ ID NO: 3 - protein, 432 aa, Lunatimonas lonarensis
SCRNSESESVRLRYADTLEAVVLDNILTKWYPAAYDYQDGGYISSFEFDFSPSERQNKMIVSQARHLWTTSKAALDYPEVDHYREGAELGFRFLRDRFWDKEHGGFHTLLSKEGEVITSGPDAKTAYGNAFAIYGLAAYYAMSNNEEVLSLAQKAFMWLEKNSYDPEFGGYFQNLGVDGTPLRRTDETPSTSTIGYKDQNSSIHLLEAFTELYHVWKDPLLKTRLEELLEIIRDKIVQPEGYLQLFLYPDFTPVSFRDSSAAVIEKHHAIDHVSYGHDVETAYLMMEASEALGRPHDEKTWAVGKKMVDHALKFGWDNEKGGFYDGGYYFKGEEIPRVVKDTKNWWAQAEGLNTLLIMADLYPDDDWGYFSKFELQWDYIDKYLIDHEHGEWYAGGIDMQPHFKTSQKGHIWKTAYHNYRSLANCIKRLREN

SEQ ID NO: 4 - DNA, 1299 bp, Lunatimonas lonarensis
tcttgcagaaattcagaaagcgaatctgtcagacttcgctatgcagatacattagaagcggttgtgctggataacatccttacaaaatggtatccggctgcctatgattatcaagatggcggatacatttcaagctttgaatttgatttttcaccgagcgaaagacaaaacaaaatgatcgtttctcaggcacgccatctttggacaacatcaaaagcagcgttagattatccggaagtggatcattatagagaaggcgcggaattaggatttcgctttctgagagatcgcttttgggataaagaacatggcggatttcatacactgctttcaaaagaaggcgaagtgatcacaagcggaccggatgctaaaacagcctatggcaatgcttttgccatttatggattagctgcctattatgctatgagcaataacgaagaagtgctttctttagcacaaaaagcgtttatgtggctggagaaaaatagctatgatccggaatttggcggatattttcagaacctgggcgtcgatggaacaccgcttagacgcacagatgaaacaccgtctacatcaacaatcggatacaaagatcagaactcttcaatccatttactggaagcgtttacagaactgtatcatgtctggaaagatccgcttttaaaaacaagacttgaagaactgcttgaaatcattcgcgataaaattgttcaaccggaaggatatctgcagctgtttctgtatccggattttacaccggtctcttttagagatagctctgcagcggttatcgaaaaacatcatgctatcgatcatgtttcatatggccatgatgtggaaacagcctatctgatgatggaagctagcgaagcccttggcagaccgcatgatgaaaaaacatgggcagtgggcaagaaaatggtcgatcatgcgcttaaatttggctgggataatgaaaaaggcggattttacgatggcggatactactttaaaggcgaagaaattccgagagtcgttaaagatacaaaaaattggtgggcacaagcggaaggattaaacacattactgatcatggctgatctgtatccggatgatgattggggctattttagcaaatttgaacttcagtgggattacatcgataaatacctgatcgatcatgaacatggagaatggtatgccggcggaatcgatatgcaaccgcattttaaaacatctcagaaaggccatatctggaaaacagcttaccataactaccgctcactggccaactgtattaaaagactgcgcgaaaattaa

SEQ ID NO: 5 - DNA, 31 bp, artificial sequence
  primer
actgctcttggatcctcttgcagaaattcag

SEQ ID NO: 6 - DNA, 30 bp, artificial sequence
  primer
gatctgcaggtcgacttaattttcgcgcag

SEQ ID NO: 7 - DNA, 20 bp, artificial sequence
  primer
gtcgacctgcagatctctag

SEQ ID NO: 8 - DNA, 17 bp, artificial sequence
  primer
ggatccaagagcagtgg

SEQ ID NO: 9 - protein, 460 aa, Melioribacter roseus
MGILKDMLNEFENNLIHKWYPLVIDKQYGGYFTNLAYDLSLMPEQEKMIVTQSRHMWTTSKAAKFLNNDTLYESALHGLNFLKNQMWDERYGGFYQIRNREGKVSDVEGWLEEKRTYGNAFAIYGLSALYELTKNNDALELAIETFNWLEERAYDPLYKGYFQFLTREGKPFGKNDSHKTNATDAVEAGYKDQNSSIHLLEAFTELYGVWRDNKVRERLEELLVLIRDKITHPKGYLQLFFERDWTPVSFRYASPEIRDANYRLDHVSFGHDYETAFLMLEASYKLGLKNDTATLYTAKKMLDHAIENGWDNSSAGFFDEGYYYSEEGECKIIKHTKNWWAQAEALNALLLFSKIFPNEKRYYKLFLQEWDYIKKYLIDHEHGDWYWGSLEKEAHYKTAPKGTIWKATYHNGRALMNCILMLSDEDSELFQSNEKFRELKSEFDDFIGHWQKTSVQAVEK

SEQ ID NO: 10 - DNA, 1383 bp, Melioribacter roseus
atgggcattctgaaagatatgcttaacgaatttgaaaacaacctgattcataaatggtatccgcttgtcatcgataaacaatatggcggatattttacaaacctggcttatgatctttcattaatgccggaacaagaaaaaatgatcgttacacagtctagacatatgtggacaacatcaaaagcagcgaaatttctgaacaacgatacactgtacgaaagcgccctgcatggacttaattttctgaaaaaccaaatgtgggatgaaagatatggcggattttatcagatcagaaatcgcgaaggcaaagtttctgatgtggaaggatggcttgaagaaaaacgcacatatggcaacgcttttgccatttatggactgtcagcactttacgaactgacaaaaaacaacgatgctctggaacttgccatcgaaacatttaattggcttgaagaaagagcgtacgatccgctgtacaaaggctactttcaatttctgacacgcgaaggcaaaccgtttggaaaaaacgatagccataaaacaaacgccacagatgcagtggaagcgggctataaagatcagaattcaagcattcatctgcttgaagcatttacagaattatatggagtgtggagagataacaaagtcagagaacgccttgaagaactgctggttctgatccgcgataaaatcacacatccgaaaggatacctgcaactgtttttcgaaagagattggacaccggtttcatttcgctatgctagcccggaaattagagatgccaattatcgcctggatcatgtgtcatttggccatgattacgaaacagcatttcttatgttagaagcgagctataaactgggacttaaaaacgatacagcaacactgtacacagcaaagaaaatgctggatcatgctatcgaaaatggctgggataactcttcagccggctttttcgatgaaggatactactacagcgaagaaggagaatgcaaaatcatcaaacatacaaaaaactggtgggcacaagcggaagctcttaacgcgcttctgctgttttctaaaatctttccgaacgaaaaaagatactacaaattatttctgcaggaatgggattacatcaaaaaatacctgatcgatcatgaacatggcgattggtattggggatctcttgaaaaagaagctcattacaaaacagccccgaaaggcacaatttggaaagcaacatatcataatggaagagcgttaatgaactgtatccttatgttaagcgatgaagattctgaactttttcagagcaacgaaaaatttcgcgaactgaaatctgaatttgatgattttatcggccattggcaaaaaacatcagtccaggctgttgaaaaataa

SEQ ID NO: 11 - DNA, 27 bp, artificial sequence
  primer
actgctcttggatccatgggcattctg

SEQ ID NO: 12 - DNA, 33 bp, artificial sequence
  primer
gatctgcaggtcgacttatttttcaacagcctg